European Patent Application EP 4 394 044 A1, published July 3, 2024. Title: METHOD FOR DETECTING FUSOBACTERIUM BACTERIUM TO DIAGNOSE ENDOMETRIOSIS. Applicant: 国立大学法人東海国立大学機構. The sequence listing filed with the application follows.

SEQUENCE LISTING (6 sequences)

SEQ ID NO: 1 - DNA, 26 bp, synthetic construct
  source 1..26: mol_type = other DNA
taggaaatacttgtaatatgaatggt

SEQ ID NO: 2 - DNA, 24 bp, synthetic construct
  source 1..24: mol_type = other DNA
gtatatccgatatcagttataggc

SEQ ID NO: 3 - DNA, 53 bp, synthetic construct
  source 1..53: mol_type = other DNA
cgaaagaactaatcccataaatacaaattggttggattaggtgtaataagtgt

SEQ ID NO: 4 - DNA, 43 bp, synthetic construct
  source 1..43: mol_type = other DNA
ggatgtgctggggtaaaaggagctgctaaaattggtatcagtg

SEQ ID NO: 5 - DNA, 44 bp, synthetic construct
  source 1..44: mol_type = other DNA
agtaatgatacaaaagttattggataaccataaatatttgaagc

SEQ ID NO: 6 - DNA, 33 bp, synthetic construct
  source 1..33: mol_type = other DNA
gtcaacagttttattacaaacatttggaatgcc